European Patent Application EP 4 656 727 A1, published December 3, 2025. Title: 核酸、重组载体、靶向整合细胞、基因表达方法和应用. Applicant: 深圳太力生物技术有限责任公司. Application CN. The sequence listing filed with the application follows.

SEQUENCE LISTING (10 sequences)

SEQ ID NO: 1 - DNA, 444 bp, synthetic construct
  source 1..444: mol_type = other DNA
taattctggcaactatcaaaggttcaccaaggaaggaattctttatttggtatctgcaagcgcctgggtgttccaatttctatctgcaaatgtttgttcctgcagacatgtctaactatggtggaaacagagaccagcctcagatgtcacactgtgacctgacctataaaagctgaactttacaaagcataagcttgggttcatgcctgagtgaaaccagactgagtttctcttgtctctccgactgcttgcttggtcctgtgctggctaaaatttccatgacagtaggggtgtaaattattcagttttagtttcccagaaaactaaaagtaagactgtcatatgacctaatgatttgacttctggggtcctttcaattagctgttgaaaggacaatagattactcatggccatttaaacaattcacagtagcaaaaaggtgag

SEQ ID NO: 2 - DNA, 2364 bp, synthetic construct
  source 1..2364: mol_type = other DNA
tcaacactcgcctctattgaagctcttggtcacgggtgaagacaggccctggtgggtcacctcgcaggcgtacactttgtgcttctcgtagtcggccttggacagggtcagggtagaggacagggagtaggtggagtccttagagtcctgttctgtcacggactcttgagagttgccagactgcagggcgttgtcgaccttccactgcaccttggcctctctagggtagaagttgttcagcaggcacacaacggaggcggtgccagatttcagctgctcgtcggaaggaggaaagatgaacacagaaggagcggccacggtccgcttgatttccagcttggttccctggccgaaggtgtagggggtctgcagagcctgcatgcagtagtaaaagcccacgtcctcagcttccactctgctgatcttcagtgtgaagtcggtgccagatccggagccggagaatctatcgggcactccgctggcccggttggagcccaggtagatcagcagctgaggggattggccgctcttctgcaggtaccaatccaggtagttgtagccgatggaatacaggaggctctgggaggaccggcaagagatagaagcaggttcgccaggggtgacaggcagagaaagtggggactgtgtcatcacgatatcacatctagcgcctctcagccacagcaggagcaggcccagcagctgagcaggcactctcatgtccatggtggcggcaagcttcgtgtcaaggacggtgactgcagaaaagacccatggaaaggaacagtctgttagtctgtcagctattatgtctggtggcgcgcgcggcagcaacgagtactgctcagactacactgccctccaccgttaacagcaccgcaacgggagttacctctgactcttatcagaacacaacaactcagctgcctgcatcttcttctgccgctgccttaagtcttccaaatgcgtcagcggtgcaagcccgctccccgagctcattttcagacacataccctaccgccacggccttgtgcggcacactggtggtggtgggcatcgtgctgtgcctaagtctggcctccactgttaggagcaaggagctgccgagcgaccatgagtcgctggaggcatgggagcagggctcggatgtagaagctccgccgctaccggagaagagcccatgtccggaacacgtacccgagattcgcgtggagatcccacgttatgtttaataaaaactgcgggcactggggacggtggtgttgtatatgtgaatttgtaaataataaatgagaccccatcctgtaaaaatacagagtccgtgtcagtctctgaaggacagtgtattggcatatagccaataaagagagttgtggcaaagagccatgttatggattagtaatggaaagtatcgtcaccaataggggagtggtcaataatggtcaataacccacacctataggctaagctataccatcacctataacatgaggaagcgggggtgtatagaccccaagccaaaaacagtatagcatgcataagaagccaagggggtgggcctatagactctataggcggtacttacgtcactcttggcacggggaatccgcgttccaatgcaccgttcccggccgcggaggctggatcggtcccggtgtcttctatggaggtcaaaacagcgtggatggcgtctccaggcgatctgacggttcactaaacgagctctgcttatatagacctcccaccgtacacgcctaccgcccatttgcgtcaatggggcggagttgttacgacattttggaaagtcccgttgattttggtgccaaaacaaactcccattgacgtcaatggggtggagacttggaaatccccgtgagtcaaaccgctatccacgcccattgatgtactgccaaaaccgcatcaccatggtaatagcgatgactaatacgtagatgtactgccaagtaggaaagtcccataaggtcatgtactgggcataatgccaggcgggccatttaccgtcattgacgtcaatagggggcgtacttggcatatgatacacttgatgtactgccaagtgggcagtttaccgtaaatactccacccattgacgtcaatggaaagtccctattggcgttactatgggaacatacgtcattattgacgtcaatgggcgggggtcgttgggcggtcagccaggcgggccatttaccgtaagttatgtaacgcggaactccatatatgggctatgaactaatgaccccgtaattgattactattaataactagtcaataatcaatgtcaacatggcggtaatgttggacatgagccaatataaatgtacatattatgatatggcggcc

SEQ ID NO: 3 - DNA, 4128 bp, synthetic construct
  source 1..4128: mol_type = other DNA
caagtaaaacctctacaaatgtggtatggctgattagccggctatcgtactcgagtcaacactcgcctctattgaagctcttggtcacgggtgaagacaggccctggtgggtcacctcgcaggcgtacactttgtgcttctcgtagtcggccttggacagggtcagggtagaggacagggagtaggtggagtccttagagtcctgttctgtcacggactcttgagagttgccagactgcagggcgttgtcgaccttccactgcaccttggcctctctagggtagaagttgttcagcaggcacacaacggaggcggtgccagatttcagctgctcgtcggaaggaggaaagatgaacacagaaggagcggccacggtccgcttgatttccagcttggttccctggccgaaggtgtagggggtctgcagagcctgcatgcagtagtaaaagcccacgtcctcagcttccactctgctgatcttcagtgtgaagtcggtgccagatccggagccggagaatctatcgggcactccgctggcccggttggagcccaggtagatcagcagctgaggggattggccgctcttctgcaggtaccaatccaggtagttgtagccgatggaatacaggaggctctgggaggaccggcaagagatagaagcaggttcgccaggggtgacaggcagagaaagtggggactgtgtcatcacgatatcacatctagcgcctctcagccacagcaggagcaggcccagcagctgagcaggcactctcatgtccatggtggcggcaagcttcgtgtcaaggacggtgactgcagaaaagacccatggaaaggaacagtctgttagtctgtcagctattatgtctggtggcgcgcgcggcagcaacgagtactgctcagactacactgccctccaccgttaacagcaccgcaacgggagttacctctgactcttatcagaacacaacaactcagctgcctgcatcttcttctgccgctgccttaagtcttccaaatgcgtcagcggtgcaagcccgctccccgagctcattttcagacacataccctaccgccacggccttgtgcggcacactggtggtggtgggcatcgtgctgtgcctaagtctggcctccactgttaggagcaaggagctgccgagcgaccatgagtcgctggaggcatgggagcagggctcggatgtagaagctccgccgctaccggagaagagcccatgtccggaacacgtacccgagattcgcgtggagatcccacgttatgtttaataaaaactgcgggcactggggacggtggtgttgtatatgtgaatttgtaaataataaatgagaccccatcctgtaaaaatacagagtccgtgtcagtctctgaaggacagtgtattggcatatagccaataaagagagttgtggcaaagagccatgttatggattagtaatggaaagtatcgtcaccaataggggagtggtcaataatggtcaataacccacacctataggctaagctataccatcacctataacatgaggaagcgggggtgtatagaccccaagccaaaaacagtatagcatgcataagaagccaagggggtgggcctatagactctataggcggtacttacgtcactcttggcacggggaatccgcgttccaatgcaccgttcccggccgcggaggctggatcggtcccggtgtcttctatggaggtcaaaacagcgtggatggcgtctccaggcgatctgacggttcactaaacgagctctgcttatatagacctcccaccgtacacgcctaccgcccatttgcgtcaatggggcggagttgttacgacattttggaaagtcccgttgattttggtgccaaaacaaactcccattgacgtcaatggggtggagacttggaaatccccgtgagtcaaaccgctatccacgcccattgatgtactgccaaaaccgcatcaccatggtaatagcgatgactaatacgtagatgtactgccaagtaggaaagtcccataaggtcatgtactgggcataatgccaggcgggccatttaccgtcattgacgtcaatagggggcgtacttggcatatgatacacttgatgtactgccaagtgggcagtttaccgtaaatactccacccattgacgtcaatggaaagtccctattggcgttactatgggaacatacgtcattattgacgtcaatgggcgggggtcgttgggcggtcagccaggcgggccatttaccgtaagttatgtaacgcggaactccatatatgggctatgaactaatgaccccgtaattgattactattaataactagtcaataatcaatgtcaacatggcggtaatgttggacatgagccaatataaatgtacatattatgatatggcggccgcatgatcctgacgacggagaccgcggtggttgaccagacaaacctacatcgcgaagcagcgcaaaacgcctaaccctaagcagattcttcatgcaattgtcggtcaagccttgccttgttgtagcttaaattttgctcgcgcactactcagcgacctccaacacacaagcagggagcagatactggcttaactatgcggcatcagagcagattgtactgagagtcgaccataggggatcgggagatctcccgatccgtcgacgtcaggtggcacttttcggggaaatgtgcgcggaacccctatttgtttatttttctaaatacattcaaatatgtatccgctcatgagacaataaccctgataaatgcttcaataatattgaaaaaggaagagtatgagtattcaacatttccgtgtcgcccttattcccttttttgcggcattttgccttcctgtttttgctcacccagaaacgctggtgaaagtaaaagatgctgaagatcagttgggtgcacgagtgggttacatcgaactggatctcaacagcggtaagatccttgagagttttcgccccgaagaacgttttccaatgatgagcacttttaaagttctgctatgtggcgcggtattatcccgtattgacgccgggcaagagcaactcggtcgccgcatacactattctcagaatgacttggttgagtactcaccagtcacagaaaagcatcttacggatggcatgacagtaagagaattatgcagtgctgccataaccatgagtgataacactgcggccaacttacttctgacaacgatcggaggaccgaaggagctaaccgcttttttgcacaacatgggggatcatgtaactcgccttgatcgttgggaaccggagctgaatgaagccataccaaacgacgagcgtgacaccacgatgcctgtagcaatggcaacaacgttgcgcaaactattaactggcgaactacttactctagcttcccggcaacaattaatagactggatggaggcggataaagttgcaggaccacttctgcgctcggcccttccggctggctggtttattgctgataaatctggagccggtgagcgtgggtctcgcggtatcattgcagcactggggccagatggtaagccctcccgtatcgtagttatctacaagagaaactcagtctggtttcactcaggcatgaacccaagcttatgctttgtaaagttcagcttttataggtcaggtcacagtgtgacatctgaggctggtctctgtttccaccatagttagacatgtctgcaggaacaaacatttgcagatagaaattggaacacccaggcgcttgcagataccaaataaagaattccttccttggtgaacctttgatagttgccagaattattccttaaggtagtttatgtgaatgtttgccttcccaagacaagaggaggggggcagagtgaactcagcacatgagtaaaacagtaactcactctgttttctaagcaatcctacagtttccaggcaggaaattctattagacaatcaaaacacagagtaatagtttgattttattaggtatgtaatatgtaagggcatatatatttcatcaccactgccaatggcagttctactatgtgtatgatcttatttcttaattatttaatttttctgtgtcttcaacacaactctactagacg

SEQ ID NO: 4 - DNA, 22 bp, synthetic construct
  source 1..22: mol_type = other DNA
agaccagcctcagatgtcacac

SEQ ID NO: 5 - DNA, 20 bp, synthetic construct
  source 1..20: mol_type = other DNA
aggcacacaacggaggcggt

SEQ ID NO: 6 - DNA, 43 bp, synthetic construct
  source 1..43: mol_type = other DNA
atgatcctgacgacggagaccgcggtggttgaccagacaaacc

SEQ ID NO: 7 - DNA, 3671 bp, synthetic construct
  source 1..3671: mol_type = other DNA
tgggtcacctcgcaggcgtacaccttgtgcttctcgtagtcggccttgctgagggtcagggtagaggacaggctgtaggtggagtccttagaatcctgctcggtgacagactcttgggagttgccggactgcagggcgttgtccaccttccactgcactttggcctctctagggtagaagttgttcagcaggcacactacagaagcggttccgctcttcagttgttcgtcagaaggagggaagatgaacacggaaggagcggccacggtccgcttgatttccactttggtgcctccgccgaaggtcagaggcaggtcccgagaatgctggcagtagtacacggcaaaatcctcgggttccagggaggagattgtcagggtgaagtcggtgccagagccgctaccggagaatctggctggcacgccggattccaggtaagaggccaggtagatcagcagccgaggggcctggccaggcttctgctggtaccagtgcagataggagtagccagaagtggacacgcccttggaggctctacaggacagtgtagccctttcgccggggctcagagacagggtagcaggagactgggtcagcacgatctcggctctgccagcccacagtagtggtagtagtagtagtagtgctcgcatggtggcggcaagcttcgtgtcaaggacggtgactgcagaaaagacccatggaaaggaacagtctgttagtctgtcagctattatgtctggtggcgcgcgcggcagcaacgagtactgctcagactacactgccctccaccgttaacagcaccgcaacgggagttacctctgactcttatcagaacacaacaactcagctgcctgcatcttcttctgccgctgccttaagtcttccaaatgcgtcagcggtgcaagcccgctccccgagctcattttcagacacataccctaccgccacggccttgtgcggcacactggtggtggtgggcatcgtgctgtgcctaagtctggcctccactgttaggagcaaggagctgccgagcgaccatgagtcgctggaggcatgggagcagggctcggatgtagaagctccgccgctaccggagaagagcccatgtccggaacacgtacccgagattcgcgtggagatcccacgttatgtttaataaaaactgcgggcactggggacggtggtgttgtatatgtgaatttgtaaataataaatgagaccccatcctgtaaaaatacagagtccgtgtcagtctctgaaggacagtgtattggcatatagccaataaagagagttgtggcaaagagccatgttatggattagtaatggaaagtatcgtcaccaataggggagtggtcaataatggtcaataacccacacctataggctaagctataccatcacctataacatgaggaagcgggggtgtatagaccccaagccaaaaacagtatagcatgcataagaagccaagggggtgggcctatagactctataggcggtacttacgtcactcttggcacggggaatccgcgttccaatgcaccgttcccggccgcggaggctggatcggtcccggtgtcttctatggaggtcaaaacagcgtggatggcgtctccaggcgatctgacggttcactaaacgagctctgcttatatagacctcccaccgtacacgcctaccgcccatttgcgtcaatggggcggagttgttacgacattttggaaagtcccgttgattttggtgccaaaacaaactcccattgacgtcaatggggtggagacttggaaatccccgtgagtcaaaccgctatccacgcccattgatgtactgccaaaaccgcatcaccatggtaatagcgatgactaatacgtagatgtactgccaagtaggaaagtcccataaggtcatgtactgggcataatgccaggcgggccatttaccgtcattgacgtcaatagggggcgtacttggcatatgatacacttgatgtactgccaagtgggcagtttaccgtaaatactccacccattgacgtcaatggaaagtccctattggcgttactatgggaacatacgtcattattgacgtcaatgggcgggggtcgttgggcggtcagccaggcgggccatttaccgtaagttatgtaacgcggaactccatatatgggctatgaactaatgaccccgtaattgattactattaataactagtcaataatcaatgtcaacatggcggtaatgttggacatgagccaatataaatgtacatattatgatatggcggccgcatgatcctgacgacggagaccgcggtggttgaccagacaaacctacatcgcgaagcagcgcaaaacgcctaaccctaagcagattcttcatgcaattgtcggtcaagccttgccttgttgtagcttaaattttgctcgcgcactactcagcgacctccaacacacaagcagggagcagatactggcttaactatgcggcatcagagcagattgtactgagagtcgaccataggggatcgggagatctcccgatccgtcgacgtcaggtggcacttttcggggaaatgtgcgcggaacccctatttgtttatttttctaaatacattcaaatatgtatccgctcatgagacaataaccctgataaatgcttcaataatattgaaaaaggaagagtatgagtattcaacatttccgtgtcgcccttattcccttttttgcggcattttgccttcctgtttttgctcacccagaaacgctggtgaaagtaaaagatgctgaagatcagttgggtgcacgagtgggttacatcgaactggatctcaacagcggtaagatccttgagagttttcgccccgaagaacgttttccaatgatgagcacttttaaagttctgctatgtggcgcggtattatcccgtattgacgccgggcaagagcaactcggtcgccgcatacactattctcagaatgacttggttgagtactcaccagtcacagaaaagcatcttacggatggcatgacagtaagagaattatgcagtgctgccataaccatgagtgataacactgcggccaacttacttctgacaacgatcggaggaccgaaggagctaaccgcttttttgcacaacatgggggatcatgtaactcgccttgatcgttgggaaccggagctgaatgaagccataccaaacgacgagcgtgacaccacgatgcctgtagcaatggcaacaacgttgcgcaaactattaactggcgaactacttactctagcttcccggcaacaattaatagactggatggaggcggataaagttgcaggaccacttctgcgctcggcccttccggctggctggtttattgctgataaatctggagccggtgagcgtgggtctcgcggtatcattgcagcactggggccagatggtaagccctcccgtatcgtagttatctacaagagaaactcagtctggtttcactcaggcatgaacccaagcttatgctttgtaaagttcagcttttataggtcaggtcacagtgtgacatctgaggctggtctctgtttccaccatagttagacatgtctgcaggaacaaacatttgcagatagaaattggaacacccaggcgcttgcagataccaaataaagaattccttcc

SEQ ID NO: 8 - DNA, 21 bp, synthetic construct
  source 1..21: mol_type = other DNA
ccttagaatcctgctcggtga

SEQ ID NO: 9 - DNA, 3131 bp, synthetic construct
  source 1..3131: mol_type = other DNA
ggtggcggtggcaagcttcgtgtcaaggacggtgactgcagaaaagacccatggaaaggaacagtctgttagtctgtcagctattatgtctggtggcgcgcgcggcagcaacgagtactgctcagactacactgccctccaccgttaacagcaccgcaacgggagttacctctgactcttatcagaacacaacaactcagctgcctgcatcttcttctgccgctgccttaagtcttccaaatgcgtcagcggtgcaagcccgctccccgagctcattttcagacacataccctaccgccacggccttgtgcggcacactggtggtggtgggcatcgtgctgtgcctaagtctggcctccactgttaggagcaaggagctgccgagcgaccatgagtcgctggaggcatgggagcagggctcggatgtagaagctccgccgctaccggagaagagcccatgtccggaacacgtacccgagattcgcgtggagatcccacgttatgtttaataaaaactgcgggcactggggacggtggtgttgtatatgtgaatttgtaaataataaatgagaccccatcctgtaaaaatacagagtccgtgtcagtctctgaaggacagtgtattggcatatagccaataaagagagttgtggcaaagagccatgttatggattagtaatggaaagtatcgtcaccaataggggagtggtcaataatggtcaataacccacacctataggctaagctataccatcacctataacatgaggaagcgggggtgtatagaccccaagccaaaaacagtatagcatgcataagaagccaagggggtgggcctatagactctataggcggtacttacgtcactcttggcacggggaatccgcgttccaatgcaccgttcccggccgcggaggctggatcggtcccggtgtcttctatggaggtcaaaacagcgtggatggcgtctccaggcgatctgacggttcactaaacgagctctgcttatatagacctcccaccgtacacgcctaccgcccatttgcgtcaatggggcggagttgttacgacattttggaaagtcccgttgattttggtgccaaaacaaactcccattgacgtcaatggggtggagacttggaaatccccgtgagtcaaaccgctatccacgcccattgatgtactgccaaaaccgcatcaccatggtaatagcgatgactaatacgtagatgtactgccaagtaggaaagtcccataaggtcatgtactgggcataatgccaggcgggccatttaccgtcattgacgtcaatagggggcgtacttggcatatgatacacttgatgtactgccaagtgggcagtttaccgtaaatactccacccattgacgtcaatggaaagtccctattggcgttactatgggaacatacgtcattattgacgtcaatgggcgggggtcgttgggcggtcagccaggcgggccatttaccgtaagttatgtaacgcggaactccatatatgggctatgaactaatgaccccgtaattgattactattaataactagtcaataatcaatgtcaacatggcggtaatgttggacatgagccaatataaatgtacatattatgatatggcggccgcatgatcctgacgacggagaccgcggtggttgaccagacaaacctacatcgcgaagcagcgcaaaacgcctaaccctaagcagattcttcatgcaattgtcggtcaagccttgccttgttgtagcttaaattttgctcgcgcactactcagcgacctccaacacacaagcagggagcagatactggcttaactatgcggcatcagagcagattgtactgagagtcgaccataggggatcgggagatctcccgatccgtcgacgtcaggtggcacttttcggggaaatgtgcgcggaacccctatttgtttatttttctaaatacattcaaatatgtatccgctcatgagacaataaccctgataaatgcttcaataatattgaaaaaggaagagtatgagtattcaacatttccgtgtcgcccttattcccttttttgcggcattttgccttcctgtttttgctcacccagaaacgctggtgaaagtaaaagatgctgaagatcagttgggtgcacgagtgggttacatcgaactggatctcaacagcggtaagatccttgagagttttcgccccgaagaacgttttccaatgatgagcacttttaaagttctgctatgtggcgcggtattatcccgtattgacgccgggcaagagcaactcggtcgccgcatacactattctcagaatgacttggttgagtactcaccagtcacagaaaagcatcttacggatggcatgacagtaagagaattatgcagtgctgccataaccatgagtgataacactgcggccaacttacttctgacaacgatcggaggaccgaaggagctaaccgcttttttgcacaacatgggggatcatgtaactcgccttgatcgttgggaaccggagctgaatgaagccataccaaacgacgagcgtgacaccacgatgcctgtagcaatggcaacaacgttgcgcaaactattaactggcgaactacttactctagcttcccggcaacaattaatagactggatggaggcggataaagttgcaggaccacttctgcgctcggcccttccggctggctggtttattgctgataaatctggagccggtgagcgtgggtctcgcggtatcattgcagcactggggccagatggtaagccctcccgtatcgtagttatctacaagagaaactcagtctggtttcactcaggcatgaacccaagcttatgctttgtaaagttcagcttttataggtcaggtcacagtgtgacatctgaggctggtctctgtttccaccatagttagacatgtctgcaggaacaaacatttgcagatagaaattggaacacccaggcgcttgcagataccaaataaagaattccttccttggtgaacctttgatagttgccagaattattccttaaggtagtttatgtgaatgtttgccttcccaagacaagaggaggggggcagagtgaactcagcacatgagtaaa

SEQ ID NO: 10 - DNA, 25 bp, synthetic construct
  source 1..25: mol_type = other DNA
tacaaatgtggtatggctgattagc